European Patent Application EP 4 800 104 A1, published September 2, 2026. Title: 一种脱氨酶、包含其的碱基编辑器及其应用. Applicant: 尧唐（上海）生物科技有限公司. Application CN. The sequence listing filed with the application follows.

SEQUENCE LISTING (47 sequences)

SEQ ID NO: 1 - protein, 170 aa, synthetic construct
MSELNDAYWMKQALALAQKAREQGEVPVGAILVLDDEVIGQGWNRAITLHDPTAHAEIMALQQGGQIVQNYRLLNATLYVTFEPCVMCAGAMVHSRIKRLVYGVSNSKRGAAGSLLNVLNYPGMNHQIEITAGVMANECSEMLCQFYQQPREVFNAEREARRLNQPDRAD

SEQ ID NO: 2 - DNA, 510 bp, synthetic construct
  source 1..510: mol_type = other DNA
atgagtgagctgaatgatgcttactggatgaaacaggcactcgctttagctcagaaggcccgggaacagggagaagttccagtgggcgctattctggtgctggatgatgaagtgataggacagggatggaatagagccatcaccctgcacgaccccaccgcccacgccgagatcatggccctgcagcagggcggccagatcgtgcagaactaccggctgctgaacgccaccctgtacgtgaccttcgagccctgcgtgatgtgcgccggcgccatggtgcacagcaggatcaagagactggtctacggcgtgagcaactcaaaaagaggcgccgccggcagcctgctgaacgtgctgaactaccccggcatgaaccaccagatcgagatcaccgccggcgtgatggccaacgagtgcagcgagatgctgtgccagttctatcagcagcctagggaagtgttcaatgctgagcgtgaggctaggcggctgaaccaacctgatagagctgac

SEQ ID NO: 3 - protein, 1609 aa, synthetic construct
MKRTADGSEFESPKKKRKVMSELNDAYWMKQALALAQKAREQGEVPVGAILVLDDEVIGQGWNRAITLHDPTAHAEIMALQQGGQIVQNYRLLNATLYVTFEPCVMCAGAMVHSRIKRLVYGVSNSKRGAAGSLLNVLNYPGMNHQIEITAGVMANECSEMLCQFYQQPREVFNAEREARRLNQPDRADSGGSSGGSSGSETPGTSESATPESSGGSSGGSDKKYSIGLAIGTNSVGWAVITDEYKVPSKKFKVLGNTDRHSIKKNLIGALLFDSGETAEATRLKRTARRRYTRRKNRICYLQEIFSNEMAKVDDSFFHRLEESFLVEEDKKHERHPIFGNIVDEVAYHEKYPTIYHLRKKLVDSTDKADLRLIYLALAHMIKFRGHFLIEGDLNPDNSDVDKLFIQLVQTYNQLFEENPINASGVDAKAILSARLSKSRRLENLIAQLPGEKKNGLFGNLIALSLGLTPNFKSNFDLAEDAKLQLSKDTYDDDLDNLLAQIGDQYADLFLAAKNLSDAILLSDILRVNTEITKAPLSASMIKRYDEHHQDLTLLKALVRQQLPEKYKEIFFDQSKNGYAGYIDGGASQEEFYKFIKPILEKMDGTEELLVKLNREDLLRKQRTFDNGSIPHQIHLGELHAILRRQEDFYPFLKDNREKIEKILTFRIPYYVGPLARGNSRFAWMTRKSEETITPWNFEEVVDKGASAQSFIERMTNFDKNLPNEKVLPKHSLLYEYFTVYNELTKVKYVTEGMRKPAFLSGEQKKAIVDLLFKTNRKVTVKQLKEDYFKKIECFDSVEISGVEDRFNASLGTYHDLLKIIKDKDFLDNEENEDILEDIVLTLTLFEDREMIEERLKTYAHLFDDKVMKQLKRRRYTGWGRLSRKLINGIRDKQSGKTILDFLKSDGFANRNFMQLIHDDSLTFKEDIQKAQVSGQGDSLHEHIANLAGSPAIKKGILQTVKVVDELVKVMGRHKPENIVIEMARENQTTQKGQKNSRERMKRIEEGIKELGSQILKEHPVENTQLQNEKLYLYYLQNGRDMYVDQELDINRLSDYDVDHIVPQSFLKDDSIDNKVLTRSDKNRGKSDNVPSEEVVKKMKNYWRQLLNAKLITQRKFDNLTKAERGGLSELDKAGFIKRQLVETRQITKHVAQILDSRMNTKYDENDKLIREVKVITLKSKLVSDFRKDFQFYKVREINNYHHAHDAYLNAVVGTALIKKYPKLESEFVYGDYKVYDVRKMIAKSEQEIGKATAKYFFYSNIMNFFKTEITLANGEIRKRPLIETNGETGEIVWDKGRDFATVRKVLSMPQVNIVKKTEVQTGGFSKESILPKRNSDKLIARKKDWDPKKYGGFDSPTVAYSVLVVAKVEKGKSKKLKSVKELLGITIMERSSFEKNPIDFLEAKGYKEVKKDLIIKLPKYSLFELENGRKRMLASAGELQKGNELALPSKYVNFLYLASHYEKLKGSPEDNEQKQLFVEQHKHYLDEIIEQISEFSKRVILADANLDKVLSAYNKHRDKPIREQAENIIHLFTLTNLGAPAAFKYFDTTIDRKRYTSTKEVLDATLIHQSITGLYETRIDLSQLGGDSGGSKRTADGSEFEPKKKRKV

SEQ ID NO: 4 - DNA, 4827 bp, synthetic construct
  source 1..4827: mol_type = other DNA
atgaaacggacagccgacggaagcgagttcgagtcaccaaagaagaagcggaaagtcatgagtgagctgaatgatgcttactggatgaaacaggcactcgctttagctcagaaggcccgggaacagggagaagttccagtgggcgctattctggtgctggatgatgaagtgataggacagggatggaatagagccatcaccctgcacgaccccaccgcccacgccgagatcatggccctgcagcagggcggccagatcgtgcagaactaccggctgctgaacgccaccctgtacgtgaccttcgagccctgcgtgatgtgcgccggcgccatggtgcacagcaggatcaagagactggtctacggcgtgagcaactcaaaaagaggcgccgccggcagcctgctgaacgtgctgaactaccccggcatgaaccaccagatcgagatcaccgccggcgtgatggccaacgagtgcagcgagatgctgtgccagttctatcagcagcctagggaagtgttcaatgctgagcgtgaggctaggcggctgaaccaacctgatagagctgactccggaggatctagcggaggctcctctggctctgagacacctggcacaagcgagagcgcaacacctgaaagcagcgggggcagcagcggggggtcagacaagaagtacagcatcggcctggccatcggcaccaactctgtgggctgggccgtgatcaccgacgagtacaaggtgcccagcaagaaattcaaggtgctgggcaacaccgaccggcacagcatcaagaagaacctgatcggagccctgctgttcgacagcggcgaaacagccgaggccacccggctgaagagaaccgccagaagaagatacaccagacggaagaaccggatctgctatctgcaagagatcttcagcaacgagatggccaaggtggacgacagcttcttccacagactggaagagtccttcctggtggaagaggataagaagcacgagcggcaccccatcttcggcaacatcgtggacgaggtggcctaccacgagaagtaccccaccatctaccacctgagaaagaaactggtggacagcaccgacaaggccgacctgcggctgatctatctggccctggcccacatgatcaagttccggggccacttcctgatcgagggcgacctgaaccccgacaacagcgacgtggacaagctgttcatccagctggtgcagacctacaaccagctgttcgaggaaaaccccatcaacgccagcggcgtggacgccaaggccatcctgtctgccagactgagcaagagcagacggctggaaaatctgatcgcccagctgcccggcgagaagaagaatggcctgttcggaaacctgattgccctgagcctgggcctgacccccaacttcaagagcaacttcgacctggccgaggatgccaaactgcagctgagcaaggacacctacgacgacgacctggacaacctgctggcccagatcggcgaccagtacgccgacctgtttctggccgccaagaacctgtccgacgccatcctgctgagcgacatcctgagagtgaacaccgagatcaccaaggcccccctgagcgcctctatgatcaagagatacgacgagcaccaccaggacctgaccctgctgaaagctctcgtgcggcagcagctgcctgagaagtacaaagagattttcttcgaccagagcaagaacggctacgccggctacattgacggcggagccagccaggaagagttctacaagttcatcaagcccatcctggaaaagatggacggcaccgaggaactgctcgtgaagctgaacagagaggacctgctgcggaagcagcggaccttcgacaacggcagcatcccccaccagatccacctgggagagctgcacgccattctgcggcggcaggaagatttttacccattcctgaaggacaaccgggaaaagatcgagaagatcctgaccttccgcatcccctactacgtgggccctctggccaggggaaacagcagattcgcctggatgaccagaaagagcgaggaaaccatcaccccctggaacttcgaggaagtggtggacaagggcgcttccgcccagagcttcatcgagcggatgaccaacttcgataagaacctgcccaacgagaaggtgctgcccaagcacagcctgctgtacgagtacttcaccgtgtataacgagctgaccaaagtgaaatacgtgaccgagggaatgagaaagcccgccttcctgagcggcgagcagaaaaaggccatcgtggacctgctgttcaagaccaaccggaaagtgaccgtgaagcagctgaaagaggactacttcaagaaaatcgagtgcttcgactccgtggaaatctccggcgtggaagatcggttcaacgcctccctgggcacataccacgatctgctgaaaattatcaaggacaaggacttcctggacaatgaggaaaacgaggacattctggaagatatcgtgctgaccctgacactgtttgaggacagagagatgatcgaggaacggctgaaaacctatgcccacctgttcgacgacaaagtgatgaagcagctgaagcggcggagatacaccggctggggcaggctgagccggaagctgatcaacggcatccgggacaagcagtccggcaagacaatcctggatttcctgaagtccgacggcttcgccaacagaaacttcatgcagctgatccacgacgacagcctgacctttaaagaggacatccagaaagcccaggtgtccggccagggcgatagcctgcacgagcacattgccaatctggccggcagccccgccattaagaagggcatcctgcagacagtgaaggtggtggacgagctcgtgaaagtgatgggccggcacaagcccgagaacatcgtgatcgaaatggccagagagaaccagaccacccagaagggacagaagaacagccgcgagagaatgaagcggatcgaagagggcatcaaagagctgggcagccagatcctgaaagaacaccccgtggaaaacacccagctgcagaacgagaagctgtacctgtactacctgcagaatgggcgggatatgtacgtggaccaggaactggacatcaaccggctgtccgactacgatgtggaccatatcgtgcctcagagctttctgaaggacgactccatcgacaacaaggtgctgaccagaagcgacaagaaccggggcaagagcgacaacgtgccctccgaagaggtcgtgaagaagatgaagaactactggcggcagctgctgaacgccaagctgattacccagagaaagttcgacaatctgaccaaggccgagagaggcggcctgagcgaactggataaggccggcttcatcaagagacagctggtggaaacccggcagatcacaaagcacgtggcacagatcctggactcccggatgaacactaagtacgacgagaatgacaagctgatccgggaagtgaaagtgatcaccctgaagtccaagctggtgtccgatttccggaaggatttccagttttacaaagtgcgcgagatcaacaactaccaccacgcccacgacgcctacctgaacgccgtcgtgggaaccgccctgatcaaaaagtaccctaagctggaaagcgagttcgtgtacggcgactacaaggtgtacgacgtgcggaagatgatcgccaagagcgagcaggaaatcggcaaggctaccgccaagtacttcttctacagcaacatcatgaactttttcaagaccgagattaccctggccaacggcgagatccggaagcggcctctgatcgagacaaacggcgaaaccggggagatcgtgtgggataagggccgggattttgccaccgtgcggaaagtgctgagcatgccccaagtgaatatcgtgaaaaagaccgaggtgcagacaggcggcttcagcaaagagtctatcctgcccaagaggaacagcgataagctgatcgccagaaagaaggactgggaccctaagaagtacggcggcttcgacagccccaccgtggcctattctgtgctggtggtggccaaagtggaaaagggcaagtccaagaaactgaagagtgtgaaagagctgctggggatcaccatcatggaaagaagcagcttcgagaagaatcccatcgactttctggaagccaagggctacaaagaagtgaaaaaggacctgatcatcaagctgcctaagtactccctgttcgagctggaaaacggccggaagagaatgctggcctctgccggcgaactgcagaagggaaacgaactggccctgccctccaaatatgtgaacttcctgtacctggccagccactatgagaagctgaagggctcccccgaggataatgagcagaaacagctgtttgtggaacagcacaagcactacctggacgagatcatcgagcagatcagcgagttctccaagagagtgatcctggccgacgctaatctggacaaagtgctgtccgcctacaacaagcaccgggataagcccatcagagagcaggccgagaatatcatccacctgtttaccctgaccaatctgggagcccctgccgccttcaagtactttgacaccaccatcgaccggaagaggtacaccagcaccaaagaggtgctggacgccaccctgatccaccagagcatcaccggcctgtacgagacacggatcgacctgtctcagctgggaggtgactctggcggctcaaaaagaaccgccgacggcagcgaattcgagcccaagaagaagaggaaagtc

SEQ ID NO: 5 - DNA, 20 bp, synthetic construct
  source 1..20: mol_type = other DNA
cccgcaccttggcgcagcgg

SEQ ID NO: 6 - DNA, 24 bp, synthetic construct
  source 1..24: mol_type = other DNA
cacccccgcaccttggcgcagcgg

SEQ ID NO: 7 - DNA, 24 bp, synthetic construct
  source 1..24: mol_type = other DNA
aaacccgctgcgccaaggtgcggg

SEQ ID NO: 8 - DNA, 20 bp, synthetic construct
  source 1..20: mol_type = other DNA
ggtgctagccttgcgttccg

SEQ ID NO: 9 - DNA, 19 bp, synthetic construct
  source 1..19: mol_type = other DNA
gtccccaagatcgtgccaa

SEQ ID NO: 10 - protein, 170 aa, synthetic construct
MSELNDAYWMKQALALAQKAREQGEVPVGAILVLDDEVIGQGWNRCYGHHDPTAHAEIMALQQGGQIVQNYRLLNATLYVTFEPCVMCAGAMVHSRIKRLVYGMSNSKRGAAGSLLNVLNYPGMNHQIEITAGVMANECSEMLCQFYQQPREVFNAEREARRLNQPDRAD

SEQ ID NO: 11 - DNA, 510 bp, synthetic construct
  source 1..510: mol_type = other DNA
atgagtgagctgaatgatgcttactggatgaaacaggcactcgctttagctcagaaggcccgggaacagggagaagttccagtgggcgctattctggtgctggatgatgaagtgataggacagggatggaatagatgctacggccatcacgaccccaccgcccacgccgagatcatggccctgcagcagggcggccagatcgtgcagaactaccggctgctgaacgccaccctgtacgtgaccttcgagccctgcgtgatgtgcgccggcgccatggtgcacagcaggatcaagagactggtctacggcatgagcaactcaaaaagaggcgccgccggcagcctgctgaacgtgctgaactaccccggcatgaaccaccagatcgagatcaccgccggcgtgatggccaacgagtgcagcgagatgctgtgccagttctatcagcagcctagggaagtgttcaatgctgagcgtgaggctaggcggctgaaccaacctgatagagctgac

SEQ ID NO: 12 - DNA, 35 bp, synthetic construct
  source 1..35: mol_type = other DNA
gaagcggaaagtcgacaagaagtacagcatcggcc

SEQ ID NO: 13 - DNA, 39 bp, synthetic construct
  source 1..39: mol_type = other DNA
ctgtacttcttgtcgactttccgcttcttctttggtgac

SEQ ID NO: 14 - DNA, 113 bp, synthetic construct
  source 1..113: mol_type = other DNA
tctggaggatctagcggcggatcctctggaagcgagacaccaggcacaagcgagtccgccacaccagagagctccggcggctcctccggaggatccagtgagctgaatgatgc

SEQ ID NO: 15 - DNA, 40 bp, synthetic construct
  source 1..40: mol_type = other DNA
tgaccccccgctgctgcccccgctgctttcaggtgttgcg

SEQ ID NO: 16 - DNA, 48 bp, synthetic construct
  source 1..48: mol_type = other DNA
ggggcagcagcggggggtcacccgaggataatgagcagaaacagctgt

SEQ ID NO: 17 - DNA, 47 bp, synthetic construct
  source 1..47: mol_type = other DNA
ccgccgctagatcctccagaggagcccttcagcttctcatagtggct

SEQ ID NO: 18 - protein, 1620 aa, synthetic construct
MKRTADGSEFESPKKKRKVMDKKYSIGLAIGTNSVGWAVITDEYKVPSKKFKVLGNTDRHSIKKNLIGALLFDSGETAEATRLKRTARRRYTRRKNRICYLQEIFSNEMAKVDDSFFHRLEESFLVEEDKKHERHPIFGNIVDEVAYHEKYPTIYHLRKKLVDSTDKADLRLIYLALAHMIKFRGHFLIEGDLNPDNSDVDKLFIQLVQTYNQLFEENPINASGVDAKAILSARLSKSRRLENLIAQLPGEKKNGLFGNLIALSLGLTPNFKSNFDLAEDAKLQLSKDTYDDDLDNLLAQIGDQYADLFLAAKNLSDAILLSDILRVNTEITKAPLSASMIKRYDEHHQDLTLLKALVRQQLPEKYKEIFFDQSKNGYAGYIDGGASQEEFYKFIKPILEKMDGTEELLVKLNREDLLRKQRTFDNGSIPHQIHLGELHAILRRQEDFYPFLKDNREKIEKILTFRIPYYVGPLARGNSRFAWMTRKSEETITPWNFEEVVDKGASAQSFIERMTNFDKNLPNEKVLPKHSLLYEYFTVYNELTKVKYVTEGMRKPAFLSGEQKKAIVDLLFKTNRKVTVKQLKEDYFKKIECFDSVEISGVEDRFNASLGTYHDLLKIIKDKDFLDNEENEDILEDIVLTLTLFEDREMIEERLKTYAHLFDDKVMKQLKRRRYTGWGRLSRKLINGIRDKQSGKTILDFLKSDGFANRNFMQLIHDDSLTFKEDIQKAQVSGQGDSLHEHIANLAGSPAIKKGILQTVKVVDELVKVMGRHKPENIVIEMARENQTTQKGQKNSRERMKRIEEGIKELGSQILKEHPVENTQLQNEKLYLYYLQNGRDMYVDQELDINRLSDYDVDHIVPQSFLKDDSIDNKVLTRSDKNRGKSDNVPSEEVVKKMKNYWRQLLNAKLITQRKFDNLTKAERGGLSELDKAGFIKRQLVETRQITKHVAQILDSRMNTKYDENDKLIREVKVITLKSKLVSDFRKDFQFYKVREINNYHHAHDAYLNAVVGTALIKKYPKLESEFVYGDYKVYDVRKMIAKSEQEIGKATAKYFFYSNIMNFFKTEITLANGEIRKRPLIETNGETGEIVWDKGRDFATVRKVLSMPQVNIVKKTEVQTGGFSKESILPKRNSDKLIARKKDWDPKKYGGFDSPTVAYSVLVVAKVEKGKSKKLKSVKELLGITIMERSSFEKNPIDFLEAKGYKEVKKDLIIKLPKYSLFELENGRKRMLASAGELQKGNELALPSKYVNFLYLASHYEKLKGSSGGSSGGSSGSETPGTSESATPESSGGSSGGSSELNDAYWMKQALALAQKAREQGEVPVGAILVLDDEVIGQGWNRCYGHHDPTAHAEIMALQQGGQIVQNYRLLNATLYVTFEPCVMCAGAMVHSRIKRLVYGMSNSKRGAAGSLLNVLNYPGMNHQIEITAGVMANECSEMLCQFYRQLRLAPGAEREARRLNQPDRADSGGSSGGSSGSETPGTSESATPESSGGSSGGSPEDNEQKQLFVEQHKHYLDEIIEQISEFSKRVILADANLDKVLSAYNKHRDKPIREQAENIIHLFTLTNLGAPAAFKYFDTTIDRKRYTSTKEVLDATLIHQSITGLYETRIDLSQLGGD

SEQ ID NO: 19 - DNA, 4860 bp, synthetic construct
  source 1..4860: mol_type = other DNA
atgaaacggacagccgacggaagcgagttcgagtcaccaaagaagaagcggaaagtcatggacaagaagtacagcatcggcctggccatcggcaccaactctgtgggctgggccgtgatcaccgacgagtacaaggtgcccagcaagaaattcaaggtgctgggcaacaccgaccggcacagcatcaagaagaacctgatcggagccctgctgttcgacagcggcgaaacagccgaggccacccggctgaagagaaccgccagaagaagatacaccagacggaagaaccggatctgctatctgcaagagatcttcagcaacgagatggccaaggtggacgacagcttcttccacagactggaagagtccttcctggtggaagaggataagaagcacgagcggcaccccatcttcggcaacatcgtggacgaggtggcctaccacgagaagtaccccaccatctaccacctgagaaagaaactggtggacagcaccgacaaggccgacctgcggctgatctatctggccctggcccacatgatcaagttccggggccacttcctgatcgagggcgacctgaaccccgacaacagcgacgtggacaagctgttcatccagctggtgcagacctacaaccagctgttcgaggaaaaccccatcaacgccagcggcgtggacgccaaggccatcctgtctgccagactgagcaagagcagacggctggaaaatctgatcgcccagctgcccggcgagaagaagaatggcctgttcggaaacctgattgccctgagcctgggcctgacccccaacttcaagagcaacttcgacctggccgaggatgccaaactgcagctgagcaaggacacctacgacgacgacctggacaacctgctggcccagatcggcgaccagtacgccgacctgtttctggccgccaagaacctgtccgacgccatcctgctgagcgacatcctgagagtgaacaccgagatcaccaaggcccccctgagcgcctctatgatcaagagatacgacgagcaccaccaggacctgaccctgctgaaagctctcgtgcggcagcagctgcctgagaagtacaaagagattttcttcgaccagagcaagaacggctacgccggctacattgacggcggagccagccaggaagagttctacaagttcatcaagcccatcctggaaaagatggacggcaccgaggaactgctcgtgaagctgaacagagaggacctgctgcggaagcagcggaccttcgacaacggcagcatcccccaccagatccacctgggagagctgcacgccattctgcggcggcaggaagatttttacccattcctgaaggacaaccgggaaaagatcgagaagatcctgaccttccgcatcccctactacgtgggccctctggccaggggaaacagcagattcgcctggatgaccagaaagagcgaggaaaccatcaccccctggaacttcgaggaagtggtggacaagggcgcttccgcccagagcttcatcgagcggatgaccaacttcgataagaacctgcccaacgagaaggtgctgcccaagcacagcctgctgtacgagtacttcaccgtgtataacgagctgaccaaagtgaaatacgtgaccgagggaatgagaaagcccgccttcctgagcggcgagcagaaaaaggccatcgtggacctgctgttcaagaccaaccggaaagtgaccgtgaagcagctgaaagaggactacttcaagaaaatcgagtgcttcgactccgtggaaatctccggcgtggaagatcggttcaacgcctccctgggcacataccacgatctgctgaaaattatcaaggacaaggacttcctggacaatgaggaaaacgaggacattctggaagatatcgtgctgaccctgacactgtttgaggacagagagatgatcgaggaacggctgaaaacctatgcccacctgttcgacgacaaagtgatgaagcagctgaagcggcggagatacaccggctggggcaggctgagccggaagctgatcaacggcatccgggacaagcagtccggcaagacaatcctggatttcctgaagtccgacggcttcgccaacagaaacttcatgcagctgatccacgacgacagcctgacctttaaagaggacatccagaaagcccaggtgtccggccagggcgatagcctgcacgagcacattgccaatctggccggcagccccgccattaagaagggcatcctgcagacagtgaaggtggtggacgagctcgtgaaagtgatgggccggcacaagcccgagaacatcgtgatcgaaatggccagagagaaccagaccacccagaagggacagaagaacagccgcgagagaatgaagcggatcgaagagggcatcaaagagctgggcagccagatcctgaaagaacaccccgtggaaaacacccagctgcagaacgagaagctgtacctgtactacctgcagaatgggcgggatatgtacgtggaccaggaactggacatcaaccggctgtccgactacgatgtggaccatatcgtgcctcagagctttctgaaggacgactccatcgacaacaaggtgctgaccagaagcgacaagaaccggggcaagagcgacaacgtgccctccgaagaggtcgtgaagaagatgaagaactactggcggcagctgctgaacgccaagctgattacccagagaaagttcgacaatctgaccaaggccgagagaggcggcctgagcgaactggataaggccggcttcatcaagagacagctggtggaaacccggcagatcacaaagcacgtggcacagatcctggactcccggatgaacactaagtacgacgagaatgacaagctgatccgggaagtgaaagtgatcaccctgaagtccaagctggtgtccgatttccggaaggatttccagttttacaaagtgcgcgagatcaacaactaccaccacgcccacgacgcctacctgaacgccgtcgtgggaaccgccctgatcaaaaagtaccctaagctggaaagcgagttcgtgtacggcgactacaaggtgtacgacgtgcggaagatgatcgccaagagcgagcaggaaatcggcaaggctaccgccaagtacttcttctacagcaacatcatgaactttttcaagaccgagattaccctggccaacggcgagatccggaagcggcctctgatcgagacaaacggcgaaaccggggagatcgtgtgggataagggccgggattttgccaccgtgcggaaagtgctgagcatgccccaagtgaatatcgtgaaaaagaccgaggtgcagacaggcggcttcagcaaagagtctatcctgcccaagaggaacagcgataagctgatcgccagaaagaaggactgggaccctaagaagtacggcggcttcgacagccccaccgtggcctattctgtgctggtggtggccaaagtggaaaagggcaagtccaagaaactgaagagtgtgaaagagctgctggggatcaccatcatggaaagaagcagcttcgagaagaatcccatcgactttctggaagccaagggctacaaagaagtgaaaaaggacctgatcatcaagctgcctaagtactccctgttcgagctggaaaacggccggaagagaatgctggcctctgccggcgaactgcagaagggaaacgaactggccctgccctccaaatatgtgaacttcctgtacctggccagccactatgagaagctgaagggctcctctggaggatctagcggcggatcctctggaagcgagacaccaggcacaagcgagtccgccacaccagagagctccggcggctcctccggaggatccagtgagctgaatgatgcttactggatgaaacaggcactcgctttagctcagaaggcccgggaacagggagaagttccagtgggcgctattctggtgctggatgatgaagtgataggacagggatggaatagatgctacggccatcacgaccccaccgcccacgccgagatcatggccctgcagcagggcggccagatcgtgcagaactaccggctgctgaacgccaccctgtacgtgaccttcgagccctgcgtgatgtgcgccggcgccatggtgcacagcaggatcaagagactggtctacggcatgagcaactcaaaaagaggcgccgccggcagcctgctgaacgtgctgaactaccccggcatgaaccaccagatcgagatcaccgccggcgtgatggccaacgagtgcagcgagatgctgtgccagttctatcgacagttgaggctcgcccccggggctgagcgtgaggctaggcggctgaaccaacctgatagagctgactccggaggatctagcggaggctcctctggctctgagacacctggcacaagcgagagcgcaacacctgaaagcagcgggggcagcagcggggggtcacccgaggataatgagcagaaacagctgtttgtggaacagcacaagcactacctggacgagatcatcgagcagatcagcgagttctccaagagagtgatcctggccgacgctaatctggacaaagtgctgtccgcctacaacaagcaccgggataagcccatcagagagcaggccgagaatatcatccacctgtttaccctgaccaatctgggagcccctgccgccttcaagtactttgacaccaccatcgaccggaagaggtacaccagcaccaaagaggtgctggacgccaccctgatccaccagagcatcaccggcctgtacgagacacggatcgacctgtctcagctgggaggtgac

SEQ ID NO: 20 - protein, 1620 aa, synthetic construct
MKRTADGSEFESPKKKRKVMDKKYSIGLAIGTNSVGWAVITDEYKVPSKKFKVLGNTDRHSIKKNLIGALLFDSGETAEATRLKRTARRRYTRRKNRICYLQEIFSNEMAKVDDSFFHRLEESFLVEEDKKHERHPIFGNIVDEVAYHEKYPTIYHLRKKLVDSTDKADLRLIYLALAHMIKFRGHFLIEGDLNPDNSDVDKLFIQLVQTYNQLFEENPINASGVDAKAILSARLSKSRRLENLIAQLPGEKKNGLFGNLIALSLGLTPNFKSNFDLAEDAKLQLSKDTYDDDLDNLLAQIGDQYADLFLAAKNLSDAILLSDILRVNTEITKAPLSASMIKRYDEHHQDLTLLKALVRQQLPEKYKEIFFDQSKNGYAGYIDGGASQEEFYKFIKPILEKMDGTEELLVKLNREDLLRKQRTFDNGSIPHQIHLGELHAILRRQEDFYPFLKDNREKIEKILTFRIPYYVGPLARGNSRFAWMTRKSEETITPWNFEEVVDKGASAQSFIERMTNFDKNLPNEKVLPKHSLLYEYFTVYNELTKVKYVTEGMRKPAFLSGEQKKAIVDLLFKTNRKVTVKQLKEDYFKKIECFDSVEISGVEDRFNASLGTYHDLLKIIKDKDFLDNEENEDILEDIVLTLTLFEDREMIEERLKTYAHLFDDKVMKQLKRRRYTGWGRLSRKLINGIRDKQSGKTILDFLKSDGFANRNFMQLIHDDSLTFKEDIQKAQVSGQGDSLHEHIANLAGSPAIKKGILQTVKVVDELVKVMGRHKPENIVIEMARENQTTQKGQKNSRERMKRIEEGIKELGSQILKEHPVENTQLQNEKLYLYYLQNGRDMYVDQELDINRLSDYDVDHIVPQSFLKDDSIDNKVLTRSDKNRGKSDNVPSEEVVKKMKNYWRQLLNAKLITQRKFDNLTKAERGGLSELDKAGFIKRQLVETRQITKHVAQILDSRMNTKYDENDKLIREVKVITLKSKLVSDFRKDFQFYKVREINNYHHAHDAYLNAVVGTALIKKYPKLESEFVYGDYKVYDVRKMIAKSEQEIGKATAKYFFYSNIMNFFKTEITLANGEIRKRPLIETNGETGEIVWDKGRDFATVRKVLSMPQVNIVKKTEVQTGGFSKESILPKRNSDKLIARKKDWDPKKYGGFDSPTVAYSVLVVAKVEKGKSKKLKSVKELLGITIMERSSFEKNPIDFLEAKGYKEVKKDLIIKLPKYSLFELENGRKRMLASAGELQKGNELALPSKYVNFLYLASHYEKLKGSSGGSSGGSSGSETPGTSESATPESSGGSSGGSSELNDAYWMKQALALAQKAREQGEVPVGAILVLDDEVIGQGWNRCYAHHDPTAHAEIMALQQGGQIVQNYRLLNATLYVTFEPCVMCAGAMVHSRIKRLVYGMSNSKRGAAGSLLNVLNYPGMNHQIEITAGVMANECSEMLCQFYRQLRLAPGAEREARRLNQPDRADSGGSSGGSSGSETPGTSESATPESSGGSSGGSPEDNEQKQLFVEQHKHYLDEIIEQISEFSKRVILADANLDKVLSAYNKHRDKPIREQAENIIHLFTLTNLGAPAAFKYFDTTIDRKRYTSTKEVLDATLIHQSITGLYETRIDLSQLGGD

SEQ ID NO: 21 - DNA, 4860 bp, synthetic construct
  source 1..4860: mol_type = other DNA
atgaaacggacagccgacggaagcgagttcgagtcaccaaagaagaagcggaaagtcatggacaagaagtacagcatcggcctggccatcggcaccaactctgtgggctgggccgtgatcaccgacgagtacaaggtgcccagcaagaaattcaaggtgctgggcaacaccgaccggcacagcatcaagaagaacctgatcggagccctgctgttcgacagcggcgaaacagccgaggccacccggctgaagagaaccgccagaagaagatacaccagacggaagaaccggatctgctatctgcaagagatcttcagcaacgagatggccaaggtggacgacagcttcttccacagactggaagagtccttcctggtggaagaggataagaagcacgagcggcaccccatcttcggcaacatcgtggacgaggtggcctaccacgagaagtaccccaccatctaccacctgagaaagaaactggtggacagcaccgacaaggccgacctgcggctgatctatctggccctggcccacatgatcaagttccggggccacttcctgatcgagggcgacctgaaccccgacaacagcgacgtggacaagctgttcatccagctggtgcagacctacaaccagctgttcgaggaaaaccccatcaacgccagcggcgtggacgccaaggccatcctgtctgccagactgagcaagagcagacggctggaaaatctgatcgcccagctgcccggcgagaagaagaatggcctgttcggaaacctgattgccctgagcctgggcctgacccccaacttcaagagcaacttcgacctggccgaggatgccaaactgcagctgagcaaggacacctacgacgacgacctggacaacctgctggcccagatcggcgaccagtacgccgacctgtttctggccgccaagaacctgtccgacgccatcctgctgagcgacatcctgagagtgaacaccgagatcaccaaggcccccctgagcgcctctatgatcaagagatacgacgagcaccaccaggacctgaccctgctgaaagctctcgtgcggcagcagctgcctgagaagtacaaagagattttcttcgaccagagcaagaacggctacgccggctacattgacggcggagccagccaggaagagttctacaagttcatcaagcccatcctggaaaagatggacggcaccgaggaactgctcgtgaagctgaacagagaggacctgctgcggaagcagcggaccttcgacaacggcagcatcccccaccagatccacctgggagagctgcacgccattctgcggcggcaggaagatttttacccattcctgaaggacaaccgggaaaagatcgagaagatcctgaccttccgcatcccctactacgtgggccctctggccaggggaaacagcagattcgcctggatgaccagaaagagcgaggaaaccatcaccccctggaacttcgaggaagtggtggacaagggcgcttccgcccagagcttcatcgagcggatgaccaacttcgataagaacctgcccaacgagaaggtgctgcccaagcacagcctgctgtacgagtacttcaccgtgtataacgagctgaccaaagtgaaatacgtgaccgagggaatgagaaagcccgccttcctgagcggcgagcagaaaaaggccatcgtggacctgctgttcaagaccaaccggaaagtgaccgtgaagcagctgaaagaggactacttcaagaaaatcgagtgcttcgactccgtggaaatctccggcgtggaagatcggttcaacgcctccctgggcacataccacgatctgctgaaaattatcaaggacaaggacttcctggacaatgaggaaaacgaggacattctggaagatatcgtgctgaccctgacactgtttgaggacagagagatgatcgaggaacggctgaaaacctatgcccacctgttcgacgacaaagtgatgaagcagctgaagcggcggagatacaccggctggggcaggctgagccggaagctgatcaacggcatccgggacaagcagtccggcaagacaatcctggatttcctgaagtccgacggcttcgccaacagaaacttcatgcagctgatccacgacgacagcctgacctttaaagaggacatccagaaagcccaggtgtccggccagggcgatagcctgcacgagcacattgccaatctggccggcagccccgccattaagaagggcatcctgcagacagtgaaggtggtggacgagctcgtgaaagtgatgggccggcacaagcccgagaacatcgtgatcgaaatggccagagagaaccagaccacccagaagggacagaagaacagccgcgagagaatgaagcggatcgaagagggcatcaaagagctgggcagccagatcctgaaagaacaccccgtggaaaacacccagctgcagaacgagaagctgtacctgtactacctgcagaatgggcgggatatgtacgtggaccaggaactggacatcaaccggctgtccgactacgatgtggaccatatcgtgcctcagagctttctgaaggacgactccatcgacaacaaggtgctgaccagaagcgacaagaaccggggcaagagcgacaacgtgccctccgaagaggtcgtgaagaagatgaagaactactggcggcagctgctgaacgccaagctgattacccagagaaagttcgacaatctgaccaaggccgagagaggcggcctgagcgaactggataaggccggcttcatcaagagacagctggtggaaacccggcagatcacaaagcacgtggcacagatcctggactcccggatgaacactaagtacgacgagaatgacaagctgatccgggaagtgaaagtgatcaccctgaagtccaagctggtgtccgatttccggaaggatttccagttttacaaagtgcgcgagatcaacaactaccaccacgcccacgacgcctacctgaacgccgtcgtgggaaccgccctgatcaaaaagtaccctaagctggaaagcgagttcgtgtacggcgactacaaggtgtacgacgtgcggaagatgatcgccaagagcgagcaggaaatcggcaaggctaccgccaagtacttcttctacagcaacatcatgaactttttcaagaccgagattaccctggccaacggcgagatccggaagcggcctctgatcgagacaaacggcgaaaccggggagatcgtgtgggataagggccgggattttgccaccgtgcggaaagtgctgagcatgccccaagtgaatatcgtgaaaaagaccgaggtgcagacaggcggcttcagcaaagagtctatcctgcccaagaggaacagcgataagctgatcgccagaaagaaggactgggaccctaagaagtacggcggcttcgacagccccaccgtggcctattctgtgctggtggtggccaaagtggaaaagggcaagtccaagaaactgaagagtgtgaaagagctgctggggatcaccatcatggaaagaagcagcttcgagaagaatcccatcgactttctggaagccaagggctacaaagaagtgaaaaaggacctgatcatcaagctgcctaagtactccctgttcgagctggaaaacggccggaagagaatgctggcctctgccggcgaactgcagaagggaaacgaactggccctgccctccaaatatgtgaacttcctgtacctggccagccactatgagaagctgaagggctcctctggaggatctagcggcggatcctctggaagcgagacaccaggcacaagcgagtccgccacaccagagagctccggcggctcctccggaggatccagtgagctgaatgatgcttactggatgaaacaggcactcgctttagctcagaaggcccgggaacagggagaagttccagtgggcgctattctggtgctggatgatgaagtgataggacagggatggaatagatgctacgcccatcacgaccccaccgcccacgccgagatcatggccctgcagcagggcggccagatcgtgcagaactaccggctgctgaacgccaccctgtacgtgaccttcgagccctgcgtgatgtgcgccggcgccatggtgcacagcaggatcaagagactggtctacggcatgagcaactcaaaaagaggcgccgccggcagcctgctgaacgtgctgaactaccccggcatgaaccaccagatcgagatcaccgccggcgtgatggccaacgagtgcagcgagatgctgtgccagttctatcgacagttgaggctcgcccccggggctgagcgtgaggctaggcggctgaaccaacctgatagagctgactccggaggatctagcggaggctcctctggctctgagacacctggcacaagcgagagcgcaacacctgaaagcagcgggggcagcagcggggggtcacccgaggataatgagcagaaacagctgtttgtggaacagcacaagcactacctggacgagatcatcgagcagatcagcgagttctccaagagagtgatcctggccgacgctaatctggacaaagtgctgtccgcctacaacaagcaccgggataagcccatcagagagcaggccgagaatatcatccacctgtttaccctgaccaatctgggagcccctgccgccttcaagtactttgacaccaccatcgaccggaagaggtacaccagcaccaaagaggtgctggacgccaccctgatccaccagagcatcaccggcctgtacgagacacggatcgacctgtctcagctgggaggtgac

SEQ ID NO: 22 - protein, 1620 aa, synthetic construct
MKRTADGSEFESPKKKRKVMDKKYSIGLAIGTNSVGWAVITDEYKVPSKKFKVLGNTDRHSIKKNLIGALLFDSGETAEATRLKRTARRRYTRRKNRICYLQEIFSNEMAKVDDSFFHRLEESFLVEEDKKHERHPIFGNIVDEVAYHEKYPTIYHLRKKLVDSTDKADLRLIYLALAHMIKFRGHFLIEGDLNPDNSDVDKLFIQLVQTYNQLFEENPINASGVDAKAILSARLSKSRRLENLIAQLPGEKKNGLFGNLIALSLGLTPNFKSNFDLAEDAKLQLSKDTYDDDLDNLLAQIGDQYADLFLAAKNLSDAILLSDILRVNTEITKAPLSASMIKRYDEHHQDLTLLKALVRQQLPEKYKEIFFDQSKNGYAGYIDGGASQEEFYKFIKPILEKMDGTEELLVKLNREDLLRKQRTFDNGSIPHQIHLGELHAILRRQEDFYPFLKDNREKIEKILTFRIPYYVGPLARGNSRFAWMTRKSEETITPWNFEEVVDKGASAQSFIERMTNFDKNLPNEKVLPKHSLLYEYFTVYNELTKVKYVTEGMRKPAFLSGEQKKAIVDLLFKTNRKVTVKQLKEDYFKKIECFDSVEISGVEDRFNASLGTYHDLLKIIKDKDFLDNEENEDILEDIVLTLTLFEDREMIEERLKTYAHLFDDKVMKQLKRRRYTGWGRLSRKLINGIRDKQSGKTILDFLKSDGFANRNFMQLIHDDSLTFKEDIQKAQVSGQGDSLHEHIANLAGSPAIKKGILQTVKVVDELVKVMGRHKPENIVIEMARENQTTQKGQKNSRERMKRIEEGIKELGSQILKEHPVENTQLQNEKLYLYYLQNGRDMYVDQELDINRLSDYDVDHIVPQSFLKDDSIDNKVLTRSDKNRGKSDNVPSEEVVKKMKNYWRQLLNAKLITQRKFDNLTKAERGGLSELDKAGFIKRQLVETRQITKHVAQILDSRMNTKYDENDKLIREVKVITLKSKLVSDFRKDFQFYKVREINNYHHAHDAYLNAVVGTALIKKYPKLESEFVYGDYKVYDVRKMIAKSEQEIGKATAKYFFYSNIMNFFKTEITLANGEIRKRPLIETNGETGEIVWDKGRDFATVRKVLSMPQVNIVKKTEVQTGGFSKESILPKRNSDKLIARKKDWDPKKYGGFDSPTVAYSVLVVAKVEKGKSKKLKSVKELLGITIMERSSFEKNPIDFLEAKGYKEVKKDLIIKLPKYSLFELENGRKRMLASAGELQKGNELALPSKYVNFLYLASHYEKLKGSSGGSSGGSSGSETPGTSESATPESSGGSSGGSSELNDAYWMKQALALAQKAREQGEVPVGAILVLDDEVIGQGWNRPITRHDPTAHAEIMALQQGGQIVQNYRLLNATLYVTFEPCVMCAGAMVHSRIKRLVYGMSNSKRGAAGSLLNVLNYPGMNHQIEITAGVMANECSEMLCQFYRQLRLAPGAEREARRLNQPDRADSGGSSGGSSGSETPGTSESATPESSGGSSGGSPEDNEQKQLFVEQHKHYLDEIIEQISEFSKRVILADANLDKVLSAYNKHRDKPIREQAENIIHLFTLTNLGAPAAFKYFDTTIDRKRYTSTKEVLDATLIHQSITGLYETRIDLSQLGGD

SEQ ID NO: 23 - DNA, 4860 bp, synthetic construct
  source 1..4860: mol_type = other DNA
atgaaacggacagccgacggaagcgagttcgagtcaccaaagaagaagcggaaagtcatggacaagaagtacagcatcggcctggccatcggcaccaactctgtgggctgggccgtgatcaccgacgagtacaaggtgcccagcaagaaattcaaggtgctgggcaacaccgaccggcacagcatcaagaagaacctgatcggagccctgctgttcgacagcggcgaaacagccgaggccacccggctgaagagaaccgccagaagaagatacaccagacggaagaaccggatctgctatctgcaagagatcttcagcaacgagatggccaaggtggacgacagcttcttccacagactggaagagtccttcctggtggaagaggataagaagcacgagcggcaccccatcttcggcaacatcgtggacgaggtggcctaccacgagaagtaccccaccatctaccacctgagaaagaaactggtggacagcaccgacaaggccgacctgcggctgatctatctggccctggcccacatgatcaagttccggggccacttcctgatcgagggcgacctgaaccccgacaacagcgacgtggacaagctgttcatccagctggtgcagacctacaaccagctgttcgaggaaaaccccatcaacgccagcggcgtggacgccaaggccatcctgtctgccagactgagcaagagcagacggctggaaaatctgatcgcccagctgcccggcgagaagaagaatggcctgttcggaaacctgattgccctgagcctgggcctgacccccaacttcaagagcaacttcgacctggccgaggatgccaaactgcagctgagcaaggacacctacgacgacgacctggacaacctgctggcccagatcggcgaccagtacgccgacctgtttctggccgccaagaacctgtccgacgccatcctgctgagcgacatcctgagagtgaacaccgagatcaccaaggcccccctgagcgcctctatgatcaagagatacgacgagcaccaccaggacctgaccctgctgaaagctctcgtgcggcagcagctgcctgagaagtacaaagagattttcttcgaccagagcaagaacggctacgccggctacattgacggcggagccagccaggaagagttctacaagttcatcaagcccatcctggaaaagatggacggcaccgaggaactgctcgtgaagctgaacagagaggacctgctgcggaagcagcggaccttcgacaacggcagcatcccccaccagatccacctgggagagctgcacgccattctgcggcggcaggaagatttttacccattcctgaaggacaaccgggaaaagatcgagaagatcctgaccttccgcatcccctactacgtgggccctctggccaggggaaacagcagattcgcctggatgaccagaaagagcgaggaaaccatcaccccctggaacttcgaggaagtggtggacaagggcgcttccgcccagagcttcatcgagcggatgaccaacttcgataagaacctgcccaacgagaaggtgctgcccaagcacagcctgctgtacgagtacttcaccgtgtataacgagctgaccaaagtgaaatacgtgaccgagggaatgagaaagcccgccttcctgagcggcgagcagaaaaaggccatcgtggacctgctgttcaagaccaaccggaaagtgaccgtgaagcagctgaaagaggactacttcaagaaaatcgagtgcttcgactccgtggaaatctccggcgtggaagatcggttcaacgcctccctgggcacataccacgatctgctgaaaattatcaaggacaaggacttcctggacaatgaggaaaacgaggacattctggaagatatcgtgctgaccctgacactgtttgaggacagagagatgatcgaggaacggctgaaaacctatgcccacctgttcgacgacaaagtgatgaagcagctgaagcggcggagatacaccggctggggcaggctgagccggaagctgatcaacggcatccgggacaagcagtccggcaagacaatcctggatttcctgaagtccgacggcttcgccaacagaaacttcatgcagctgatccacgacgacagcctgacctttaaagaggacatccagaaagcccaggtgtccggccagggcgatagcctgcacgagcacattgccaatctggccggcagccccgccattaagaagggcatcctgcagacagtgaaggtggtggacgagctcgtgaaagtgatgggccggcacaagcccgagaacatcgtgatcgaaatggccagagagaaccagaccacccagaagggacagaagaacagccgcgagagaatgaagcggatcgaagagggcatcaaagagctgggcagccagatcctgaaagaacaccccgtggaaaacacccagctgcagaacgagaagctgtacctgtactacctgcagaatgggcgggatatgtacgtggaccaggaactggacatcaaccggctgtccgactacgatgtggaccatatcgtgcctcagagctttctgaaggacgactccatcgacaacaaggtgctgaccagaagcgacaagaaccggggcaagagcgacaacgtgccctccgaagaggtcgtgaagaagatgaagaactactggcggcagctgctgaacgccaagctgattacccagagaaagttcgacaatctgaccaaggccgagagaggcggcctgagcgaactggataaggccggcttcatcaagagacagctggtggaaacccggcagatcacaaagcacgtggcacagatcctggactcccggatgaacactaagtacgacgagaatgacaagctgatccgggaagtgaaagtgatcaccctgaagtccaagctggtgtccgatttccggaaggatttccagttttacaaagtgcgcgagatcaacaactaccaccacgcccacgacgcctacctgaacgccgtcgtgggaaccgccctgatcaaaaagtaccctaagctggaaagcgagttcgtgtacggcgactacaaggtgtacgacgtgcggaagatgatcgccaagagcgagcaggaaatcggcaaggctaccgccaagtacttcttctacagcaacatcatgaactttttcaagaccgagattaccctggccaacggcgagatccggaagcggcctctgatcgagacaaacggcgaaaccggggagatcgtgtgggataagggccgggattttgccaccgtgcggaaagtgctgagcatgccccaagtgaatatcgtgaaaaagaccgaggtgcagacaggcggcttcagcaaagagtctatcctgcccaagaggaacagcgataagctgatcgccagaaagaaggactgggaccctaagaagtacggcggcttcgacagccccaccgtggcctattctgtgctggtggtggccaaagtggaaaagggcaagtccaagaaactgaagagtgtgaaagagctgctggggatcaccatcatggaaagaagcagcttcgagaagaatcccatcgactttctggaagccaagggctacaaagaagtgaaaaaggacctgatcatcaagctgcctaagtactccctgttcgagctggaaaacggccggaagagaatgctggcctctgccggcgaactgcagaagggaaacgaactggccctgccctccaaatatgtgaacttcctgtacctggccagccactatgagaagctgaagggctcctctggaggatctagcggcggatcctctggaagcgagacaccaggcacaagcgagtccgccacaccagagagctccggcggctcctccggaggatccagtgagctgaatgatgcttactggatgaaacaggcactcgctttagctcagaaggcccgggaacagggagaagttccagtgggcgctattctggtgctggatgatgaagtgataggacagggatggaatagacccatcacccggcacgaccccaccgcccacgccgagatcatggccctgcagcagggcggccagatcgtgcagaactaccggctgctgaacgccaccctgtacgtgaccttcgagccctgcgtgatgtgcgccggcgccatggtgcacagcaggatcaagagactggtctacggcatgagcaactcaaaaagaggcgccgccggcagcctgctgaacgtgctgaactaccccggcatgaaccaccagatcgagatcaccgccggcgtgatggccaacgagtgcagcgagatgctgtgccagttctatcgacagttgaggctcgcccccggggctgagcgtgaggctaggcggctgaaccaacctgatagagctgactccggaggatctagcggaggctcctctggctctgagacacctggcacaagcgagagcgcaacacctgaaagcagcgggggcagcagcggggggtcacccgaggataatgagcagaaacagctgtttgtggaacagcacaagcactacctggacgagatcatcgagcagatcagcgagttctccaagagagtgatcctggccgacgctaatctggacaaagtgctgtccgcctacaacaagcaccgggataagcccatcagagagcaggccgagaatatcatccacctgtttaccctgaccaatctgggagcccctgccgccttcaagtactttgacaccaccatcgaccggaagaggtacaccagcaccaaagaggtgctggacgccaccctgatccaccagagcatcaccggcctgtacgagacacggatcgacctgtctcagctgggaggtgac

SEQ ID NO: 24 - protein, 18 aa, synthetic construct
KRTADGSEFESPKKKRKV

SEQ ID NO: 25 - protein, 20 aa, synthetic construct
AVKRPAATKKAGQAKKKKLD

SEQ ID NO: 26 - protein, 16 aa, synthetic construct
KRPAATKKAGQAKKKK

SEQ ID NO: 27 - protein, 17 aa, synthetic construct
KKTELQTTNAENKTKKL

SEQ ID NO: 28 - protein, 19 aa, synthetic construct
KRGINDRNFWRGENGRKTR

SEQ ID NO: 29 - protein, 16 aa, synthetic construct
RKSGKIAAIVVKRPRK

SEQ ID NO: 30 - protein, 7 aa, synthetic construct
PKKKRKV

SEQ ID NO: 31 - protein, 30 aa, synthetic construct
MDSLLMNRRKFLYQFKNVRWAKGRRETYLC

SEQ ID NO: 32 - protein, 5 aa, synthetic construct
GGGGS

SEQ ID NO: 33 - protein, 4 aa, synthetic construct
SGGS

SEQ ID NO: 34 - protein, 24 aa, synthetic construct
SGGSSGSETPGTSESATPESSGGS

SEQ ID NO: 35 - protein, 32 aa, synthetic construct
SGGSSGGSSGSETPGTSESATPESSGGSSGGS

SEQ ID NO: 36 - protein, 104 aa, synthetic construct
GGSGGSPGSPAGSPTSTEEGTSESATPESGPGTSTEPSEGSAPGSPAGSPTSTEEGTSTEPSEGSAPGTSTEPSEGSAPGTSESATPESGPGSEPATSGGSGGS

SEQ ID NO: 37 - protein, 16 aa, synthetic construct
SGSETPGTSESATPES

SEQ ID NO: 38 - protein, 24 aa, synthetic construct
SGGSSGGSSGSETPGTSESATPES

SEQ ID NO: 39 - protein, 40 aa, synthetic construct
SGGSSGGSSGSETPGTSESATPESSGGSSGGSSGGSSGGS

SEQ ID NO: 40 - protein, 64 aa, synthetic construct
SGGSSGGSSGSETPGTSESATPESSGGSSGGSSGGSSGGSSGSETPGTSESATPESSGGSSGGS

SEQ ID NO: 41 - protein, 92 aa, synthetic construct
PGSPAGSPTSTEEGTSESATPESGPGTSTEPSEGSAPGSPAGSPTSTEEGTSTEPSEGSAPGTSTEPSEGSAPGTSESATPESGPGSEPATS

SEQ ID NO: 42 - DNA, 20 bp, synthetic construct
  source 1..20: mol_type = other DNA
atcgacaagaaagggactga

SEQ ID NO: 43 - DNA, 20 bp, synthetic construct
  source 1..20: mol_type = other DNA
gacagggagggagaggatgt

SEQ ID NO: 44 - DNA, 20 bp, synthetic construct
  source 1..20: mol_type = other DNA
acagcactgttacctggagc

SEQ ID NO: 45 - DNA, 20 bp, synthetic construct
  source 1..20: mol_type = other DNA
acttctccacaggagtcaga

SEQ ID NO: 46 - DNA, 20 bp, synthetic construct
  source 1..20: mol_type = other DNA
taagccagtgccagaagagc

SEQ ID NO: 47 - DNA, 20 bp, synthetic construct
  source 1..20: mol_type = other DNA
atagaccaataggcagagag